European Patent Application EP 4 273 157 A1, published November 8, 2023. Title: IMMUNOGLOBULIN-BINDING PROTEIN VARIANTS WITH INCREASED ALKALI-TOLERANCE AND USE THEREOF. Applicant: AMICOGEN, INC. The sequence listing filed with the application follows.

SEQUENCE LISTING (50 sequences)

SEQ ID NO: 1 - DNA, 756 bp, synthetic construct
  misc_feature 1..756: note = Synthetic_Herceptin scFv coding nucleic acid sequence
  source 1..756: mol_type = other DNA
aagcttgatattcagatgacccagagcccgtccagcctgtcagcaagcgttggcgaccgtgttacgattacctgccgtgcctcgcaagatgtgaacaccgcggtggcctggtatcagcaaaaaccgggcaaagcaccgaaactgctgatttatagtgcttcctttctgtactctggtgttccgtcccgtttctcaggctcgcgcagcggtaccgattttaccctgacgatcagctctctgcagccggaagacttcgccacgtattactgccagcaacactacacgaccccgccgaccttcggccagggcaccaaagtggaaatcaaaggcgccagcggcggtggcggttctggtggcggtggcagcggtggcggtggctcaagcgaagtccaactggtcgaatcgggtggtggtctggttcagccgggcggttcactgcgtctgtcgtgtgctgcctcgggtttcaacatcaaagatacctatattcattgggtgcgtcaggccccgggtaaaggtctggaatgggttgcccgcatctacccgaccaacggctatacgcgttacgccgatagcgttaaaggtcgctttaccatttctgcagacaccagtaaaaacacggcttatctgcagatgaactctctgcgtgcggaagacacggccgtgtattactgcagtcgctggggcggtgatggcttttatgcaatggactactggggccagggtaccctggttacggtcagctctggctccgagctc

SEQ ID NO: 2 - protein, 252 aa, synthetic construct
  REGION 1..252: note = Synthetic_Herceptin scFv amino acid sequence
KLDIQMTQSPSSLSASVGDRVTITCRASQDVNTAVAWYQQKPGKAPKLLIYSASFLYSGVPSRFSGSRSGTDFTLTISSLQPEDFATYYCQQHYTTPPTFGQGTKVEIKGASGGGGSGGGGSGGGGSSEVQLVESGGGLVQPGGSLRLSCAASGFNIKDTYIHWVRQAPGKGLEWVARIYPTNGYTRYADSVKGRFTISADTSKNTAYLQMNSLRAEDTAVYYCSRWGGDGFYAMDYWGQGTLVTVSSGSEL

SEQ ID NO: 3 - DNA, 219 bp, synthetic construct
  misc_feature 1..219: note = Synthetic_Wild-type Protein L B3 domain coding nucleic acid sequence
  source 1..219: mol_type = other DNA
atgccgaaagaagaggttactattaaggctaatctgatttacgccgacggaaaaacccagaccgctgagttcaagggtacttttgaagaagcgacggcagaggcgtatcggtacgcagatctgttagcgaaagaaaatggtaagtatactgtagacgttgccgacaaggggtataccttaaatatcaagttcgcaggtaaagagaaaaccccggaagaa

SEQ ID NO: 4 - protein, 73 aa, synthetic construct
  REGION 1..73: note = Synthetic_Wild-type Protein L B3 domain amino acid sequence
MPKEEVTIKANLIYADGKTQTAEFKGTFEEATAEAYRYADLLAKENGKYTVDVADKGYTLNIKFAGKEKTPEE

SEQ ID NO: 5 - DNA, 20 bp, synthetic construct
  misc_feature 1..20: note = Synthetic_EP-F error prone pcr forward primer
  source 1..20: mol_type = other DNA
gcttgatatcgaattcctgc

SEQ ID NO: 6 - DNA, 20 bp, synthetic construct
  misc_feature 1..20: note = Synthetic_T7 primer
  source 1..20: mol_type = other DNA
taatacgactcactataggg

SEQ ID NO: 7 - protein, 73 aa, synthetic construct
  REGION 1..73: note = Synthetic_Protein L B3 domain variant EP1(E28A)
MPKEEVTIKANLIYADGKTQTAEFKGTFAEATAEAYRYADLLAKENGKYTVDVADKGYTLNIKFAGKEKTPEE

SEQ ID NO: 8 - protein, 73 aa, synthetic construct
  REGION 1..73: note = Synthetic_Protein L B3 domain variant EP2(E28G)
MPKEEVTIKANLIYADGKTQTAEFKGTFGEATAEAYRYADLLAKENGKYTVDVADKGYTLNIKFAGKEKTPEE

SEQ ID NO: 9 - protein, 73 aa, synthetic construct
  REGION 1..73: note = Synthetic_Protein L B3 domain variant BEP1(E28G/Y13F)
MPKEEVTIKANLIFADGKTQTAEFKGTFGEATAEAYRYADLLAKENGKYTVDVADKGYTLNIKFAGKEKTPEE

SEQ ID NO: 10 - protein, 73 aa, synthetic construct
  REGION 1..73: note = Synthetic_Protein L B3 domain variant (E28G/K43P)
MPKEEVTIKANLIYADGKTQTAEFKGTFGEATAEAYRYADLLAPENGKYTVDVADKGYTLNIKFAGKEKTPEE

SEQ ID NO: 11 - protein, 73 aa, synthetic construct
  REGION 1..73: note = Synthetic_Protein L B3 domain variant BEP3(E28G/D51V)
MPKEEVTIKANLIYADGKTQTAEFKGTFGEATAEAYRYADLLAKENGKYTVVVADKGYTLNIKFAGKEKTPEE

SEQ ID NO: 12 - protein, 73 aa, synthetic construct
  REGION 1..73: note = Synthetic_Protein L B3 domain variant BEP4(E28G/N60E)
MPKEEVTIKANLIYADGKTQTAEFKGTFGEATAEAYRYADLLAKENGKYTVDVADKGYTLEIKFAGKEKTPEE

SEQ ID NO: 13 - DNA, 49 bp, synthetic construct
  misc_feature 1..49: note = Synthetic_28-F primer, wherein n is A, T, G, or C, and k is G or T
  source 1..49: mol_type = other DNA
gaccgctgagttcaagggtacttttnnkgaagcgacggcagaggcgtat

SEQ ID NO: 14 - DNA, 49 bp, synthetic construct
  misc_feature 1..49: note = Synthetic_28-R primer, wherein n is A, T, G, or C, and m is A or C
  source 1..49: mol_type = other DNA
atacgcctctgccgtcgcttcmnnaaaagtacccttgaactcagcggtc

SEQ ID NO: 15 - DNA, 45 bp, synthetic construct
  misc_feature 1..45: note = Synthetic_13-F primer, wherein n is A, T, G, or C, and k is G or T
  source 1..45: mol_type = other DNA
ggttactattaaggctaatctgattnnkgccgacggaaaaaccca

SEQ ID NO: 16 - DNA, 45 bp, synthetic construct
  misc_feature 1..45: note = Synthetic_13-R primer, wherein n is A, T, G, or C, and m is A or C
  source 1..45: mol_type = other DNA
tgggtttttccgtcggcmnnaatcagattagccttaatagtaacc

SEQ ID NO: 17 - DNA, 46 bp, synthetic construct
  misc_feature 1..46: note = Synthetic_43-F primer, wherein n is A, T, G, or C, and k is G or T
  source 1..46: mol_type = other DNA
gtacgcagatctgttagcgnnkgaatatggtaagtatactgtagcg

SEQ ID NO: 18 - DNA, 47 bp, synthetic construct
  misc_feature 1..47: note = Synthetic_43-R primer, wherein n is A, T, G, or C, and m is A or C
  source 1..47: mol_type = other DNA
cgtctacagtatacttaccatattcmnncgctaacagatctgcgtac

SEQ ID NO: 19 - DNA, 47 bp, synthetic construct
  misc_feature 1..47: note = Synthetic_51-F primer, wherein n is A, T, G, or C, and k is G or T
  source 1..47: mol_type = other DNA
gcgaaagaatatggtaagtatactgtannkgttgccgacaaggggta

SEQ ID NO: 20 - DNA, 47 bp, synthetic construct
  misc_feature 1..47: note = Synthetic_51-R primer, wherein n is A, T, G, or C, and m is A or C
  source 1..47: mol_type = other DNA
taccccttgtcggcaacmnntacagtatacttaccatattctttcgc

SEQ ID NO: 21 - DNA, 44 bp, synthetic construct
  misc_feature 1..44: note = Synthetic_60-F primer, wherein n is A, T, G, or C, and k is G or T
  source 1..44: mol_type = other DNA
ccgacaaggggtataccttannkatcaagttcgcaggtaaagag

SEQ ID NO: 22 - DNA, 44 bp, synthetic construct
  misc_feature 1..44: note = Synthetic_60-R primer, wherein n is A, T, G, or C, and m is A or C
  source 1..44: mol_type = other DNA
ctctttacctgcgagcttgatmnntaaggtataccccttgtcgg

SEQ ID NO: 23 - protein, 73 aa, synthetic construct
  REGION 1..73: note = Synthetic_Protein L B3 domain variant EPS1(E28L)
MPKEEVTIKANLIYADGKTQTAEFKGTFLEATAEAYRYADLLAKENGKYTVDVADKGYTLNIKFAGKEKTPEE

SEQ ID NO: 24 - protein, 73 aa, synthetic construct
  REGION 1..73: note = Synthetic_Protein L B3 domain variant EPS2(E28P)
MPKEEVTIKANLIYADGKTQTAEFKGTFPEATAEAYRYADLLAKENGKYTVDVADKGYTLNIKFAGKEKTPEE

SEQ ID NO: 25 - protein, 73 aa, synthetic construct
  REGION 1..73: note = Synthetic_Protein L B3 domain variant EPS3(E28W)
MPKEEVTIKANLIYADGKTQTAEFKGTFWEATAEAYRYADLLAKENGKYTVDVADKGYTLNIKFAGKEKTPEE

SEQ ID NO: 26 - protein, 73 aa, synthetic construct
  REGION 1..73: note = Synthetic_Protein L B3 domain variant EPS4(E28G/K43E)
MPKEEVTIKANLIYADGKTQTAEFKGTFGEATAEAYRYADLLAEENGKYTVDVADKGYTLNIKFAGKEKTPEE

SEQ ID NO: 27 - protein, 73 aa, synthetic construct
  REGION 1..73: note = Synthetic_Protein L B3 domain variant EPS5(E28G/D51T)
MPKEEVTIKANLIYADGKTQTAEFKGTFGEATAEAYRYADLLAKENGKYTVTVADKGYTLNIKFAGKEKTPEE

SEQ ID NO: 28 - protein, 73 aa, synthetic construct
  REGION 1..73: note = Synthetic_Protein L B3 domain variant EPS6(E28G/N60F)
MPKEEVTIKANLIYADGKTQTAEFKGTFGEATAEAYRYADLLAKENGKYTVDVADKGYTLFIKFAGKEKTPEE

SEQ ID NO: 29 - DNA, 48 bp, synthetic construct
  misc_feature 1..48: note = Synthetic_SH13-F1 primer
  source 1..48: mol_type = other DNA
ggttactattaaggctaatctgatttacgccgacggaaaaacccagac

SEQ ID NO: 30 - DNA, 48 bp, synthetic construct
  misc_feature 1..48: note = Synthetic_SH13-F2 primer
  source 1..48: mol_type = other DNA
ggttactattaaggctaatctgattgaggccgacggaaaaacccagac

SEQ ID NO: 31 - DNA, 48 bp, synthetic construct
  misc_feature 1..48: note = Synthetic_SH13-R1 primer
  source 1..48: mol_type = other DNA
gtctgggtttttccgtcggcgtaaatcagattagccttaatagtaacc

SEQ ID NO: 32 - DNA, 48 bp, synthetic construct
  misc_feature 1..48: note = Synthetic_SH13-R2 primer
  source 1..48: mol_type = other DNA
gtctgggtttttccgtcggcctcaatcagattagccttaatagtaacc

SEQ ID NO: 33 - DNA, 47 bp, synthetic construct
  misc_feature 1..47: note = Synthetic_SH43-F1 primer, wherein r is G or A
  source 1..47: mol_type = other DNA
cgcagatctgttagcgaaagaaraaggtaagtatactgtagacgttg

SEQ ID NO: 34 - DNA, 47 bp, synthetic construct
  misc_feature 1..47: note = Synthetic_SH43-F2 primer
  source 1..47: mol_type = other DNA
cgcagatctgttagcgaaagaaccaggtaagtatactgtagacgttg

SEQ ID NO: 35 - DNA, 47 bp, synthetic construct
  misc_feature 1..47: note = Synthetic_SH43-R1 primer, wherein y is C or T
  source 1..47: mol_type = other DNA
caacgtctacagtatacttaccttyttctttcgctaacagatctgcg

SEQ ID NO: 36 - DNA, 47 bp, synthetic construct
  misc_feature 1..47: note = Synthetic_SH43-R2 primer
  source 1..47: mol_type = other DNA
caacgtctacagtatacttacctggttctttcgctaacagatctgcg

SEQ ID NO: 37 - DNA, 54 bp, synthetic construct
  misc_feature 1..54: note = Synthetic_SH51-F1 primer, wherein w is A or T
  source 1..54: mol_type = other DNA
gcgaaagaatatggtaagtatactgtagwcgttgccgacaaggggtatacctta

SEQ ID NO: 38 - DNA, 54 bp, synthetic construct
  misc_feature 1..54: note = Synthetic_SH51-F2 primer
  source 1..54: mol_type = other DNA
gcgaaagaatatggtaagtatactgtaaccgttgccgacaaggggtatacctta

SEQ ID NO: 39 - DNA, 54 bp, synthetic construct
  misc_feature 1..54: note = Synthetic_SH51-R1 primer, wherein w is A or T
  source 1..54: mol_type = other DNA
taaggtataccccttgtcggcaacgwctacagtatacttaccatattctttcgc

SEQ ID NO: 40 - DNA, 47 bp, synthetic construct; identical to SEQ ID NO: 36
  misc_feature 1..47: note = Synthetic_SH51-R2 primer
  source 1..47: mol_type = other DNA

SEQ ID NO: 41 - DNA, 45 bp, synthetic construct
  misc_feature 1..45: note = Synthetic_SH60-F1 primer
  source 1..45: mol_type = other DNA
gccgacaaggggtataccttaaatatcaagttcgcaggtaaagag

SEQ ID NO: 42 - DNA, 45 bp, synthetic construct
  misc_feature 1..45: note = Synthetic_SH60-F2 primer
  source 1..45: mol_type = other DNA
gccgacaaggggtataccttagagatcaagttcgcaggtaaagag

SEQ ID NO: 43 - DNA, 45 bp, synthetic construct
  misc_feature 1..45: note = Synthetic_SH60-F3 primer
  source 1..45: mol_type = other DNA
gccgacaaggggtataccttatttatcaagttcgcaggtaaagag

SEQ ID NO: 44 - DNA, 45 bp, synthetic construct
  misc_feature 1..45: note = Synthetic_SH60-R1 primer
  source 1..45: mol_type = other DNA
ctctttacctgcgaacttgatatttaaggtataccccttgtcggc

SEQ ID NO: 45 - DNA, 45 bp, synthetic construct
  misc_feature 1..45: note = Synthetic_SH60-R2 primer
  source 1..45: mol_type = other DNA
ctctttacctgcgaacttgatctctaaggtataccccttgtcggc

SEQ ID NO: 46 - DNA, 45 bp, synthetic construct
  misc_feature 1..45: note = Synthetic_SH60-R3 primer
  source 1..45: mol_type = other DNA
ctctttacctgcgaacttgataaataaggtataccccttgtcggc

SEQ ID NO: 47 - protein, 73 aa, synthetic construct
  REGION 1..73: note = Synthetic_Protein L B3 domain variant mBF (Y13F/E28G/K43P)
MPKEEVTIKANLIFADGKTQTAEFKGTFGEATAEAYRYADLLAPENGKYTVDVADKGYTLNIKFAGKEKTPEE

SEQ ID NO: 48 - DNA, 876 bp, synthetic construct
  misc_feature 1..876: note = Synthetic_Protein L B3 domain variant mBF repeat (4mBF) coding nucleic acid sequence
  source 1..876: mol_type = other DNA
atgccgaaagaagaggttactattaaggctaatctgattttcgccgacggaaaaacccagaccgctgagttcaagggtacttttggggaagcgacggcagaggcgtatcggtacgcagatctgttagcgccagaaaatggtaagtatactgtagacgttgccgacaaggggtataccttaaatatcaagttcgcaggtaaagagaaaaccccggaagaaatgccgaaagaagaggttactattaaggctaatctgattttcgccgacggaaaaacccagaccgctgagttcaagggtacttttggggaagcgacggcagaggcgtatcggtacgcagatctgttagcgccagaaaatggtaagtatactgtagacgttgccgacaaggggtataccttaaatatcaagttcgcaggtaaagagaaaaccccggaagaaatgccgaaagaagaggttactattaaggctaatctgattttcgccgacggaaaaacccagaccgctgagttcaagggtacttttggggaagcgacggcagaggcgtatcggtacgcagatctgttagcgccagaaaatggtaagtatactgtagacgttgccgacaaggggtataccttaaatatcaagttcgcaggtaaagagaaaaccccggaagaaatgccgaaagaagaggttactattaaggctaatctgattttcgccgacggaaaaacccagaccgctgagttcaagggtacttttggggaagcgacggcagaggcgtatcggtacgcagatctgttagcgccagaaaatggtaagtatactgtagacgttgccgacaaggggtataccttaaatatcaagttcgcaggtaaagagaaaaccccggaagaa

SEQ ID NO: 49 - protein, 292 aa, synthetic construct
  REGION 1..292: note = Synthetic_Protein L B3 domain variant mBF repeat (4mBF)
MPKEEVTIKANLIFADGKTQTAEFKGTFGEATAEAYRYADLLAPENGKYTVDVADKGYTLNIKFAGKEKTPEEMPKEEVTIKANLIFADGKTQTAEFKGTFGEATAEAYRYADLLAPENGKYTVDVADKGYTLNIKFAGKEKTPEEMPKEEVTIKANLIFADGKTQTAEFKGTFGEATAEAYRYADLLAPENGKYTVDVADKGYTLNIKFAGKEKTPEEMPKEEVTIKANLIFADGKTQTAEFKGTFGEATAEAYRYADLLAPENGKYTVDVADKGYTLNIKFAGKEKTPEE

SEQ ID NO: 50 - protein, 719 aa, synthetic construct
  REGION 1..719: note = Synthetic_Protein L (AAA25612.1), wherein 1..18 region is a signal peptide
MAALAGAIVVTGGVGSYAADEPIDLEKLEEKRDKENVGNLPKFDNEVKDGSENPMAKYPDFDDEASTRFETENNEFEEKKVVSDNFFDQSEHPFVENKEETPETPETDSEEEVTIKANLIFANGSTQTAEFKGTFEKATSEAYAYADTLKKDNGEYTVDVADKGYTLNIKFAGKEKTPEEPKEEVTIKANLIYADGKTQTAEFKGTFEEATAEAYRYADALKKDNGEYTVDVADKGYTLNIKFAGKEKTPEEPKEEVTIKANLIYADGKTQTAEFKGTFEEATAEAYRYADLLAKENGKYTVDVADKGYTLNIKFAGKEKTPEEPKEEVTIKANLIYADGKTQTAEFKGTFAEATAEAYRYADLLAKENGKYTADLEDGGYTINIRFAGKKVDEKPEEKEQVTIKENIYFEDGTVQTATFKGTFAEATAEAYRYADLLSKEHGKYTADLEDGGYTINIRFAGKEEPEETPEKPEVQDGYASYEEAEAAAKEALKNDDVNKSYTIRQGADGRYYYVLSPVEAEEEKPEAQNGYATYEEAEAAAKKALENDPINKSYSIRQGADGRYYYVLSPVEAETPEKPVEPSEPSTPDVPSNPSNPSTPDVPSTPDVPSNPSTPEVPSNPSTPGNEEKPGNEQKPGNEQKPGNEQKPGNEQKPGNEQKPDQPSKPEKEENGKGGVDSPKKKEKAALPKAGSEAEILTLAAASLSSVAGAFISLKKRK